European Patent Application EP 4 219 539 A1, published August 2, 2023. Title: GLP-1R/GCGR Dual Target Agonist Polypeptide Derivative for Treatment of Hepatic Fibrosis Associated with Viral Hepatitis. Applicant: Shenzhen Turier Biotech. Co., Ltd. The sequence listing filed with the application follows.

SEQUENCE LISTING (26 sequences)

SEQ ID NO: 1 - protein, 40 aa, Artificial Sequence
  Polypeptide compound
  MISC_FEATURE (2)..(2): X=D-Ser
  MISC_FEATURE (16)..(16): A side chain of Lys is linked to -PEG2-PEG2-γGlu-CO(CH2)14CH3
HXQGTFTSDYSKYLDKRRAQDFVQWLMNTGGPSSGAPPPS

SEQ ID NO: 2 - protein, 40 aa, Artificial Sequence
  Polypeptide compound
  MISC_FEATURE (2)..(2): Xaa=D-Ser
  MISC_FEATURE (17)..(17): A side chain of Lys is linked to -PEG2-PEG2-γGlu-CO(CH2)16CO2H
HXQGTFTSDYSKYLDEKRAQDFVQWLMNTGGPSSGAPPPS

SEQ ID NO: 3 - protein, 40 aa, Artificial Sequence
  Polypeptide compound
  MISC_FEATURE (2)..(2): Aib
  MISC_FEATURE (10)..(10): A side chain of Lys is linked to -PEG2-PEG2-γGlu-CO(CH2)14CO2H
HXQGTFTSDKSKYLDERRAQDFVQWLLDGGGPSSGAPPPS

SEQ ID NO: 4 - protein, 39 aa, Artificial Sequence
  Polypeptide compound
  MISC_FEATURE (2)..(2): Xaa=Aib
  MISC_FEATURE (10)..(10): A side chain of Lys is linked to -PEG2-PEG2-γGlu-CO(CH2)16CH3
HXQGTFTSDKSKYLDERRAQDFVQWLLDGGPSSGAPPPS

SEQ ID NO: 5 - protein, 40 aa, Artificial Sequence; identical to SEQ ID NO: 3
  Polypeptide compound
  MISC_FEATURE (2)..(2): Xaa=Aib
  MISC_FEATURE (10)..(10): A side chain of Lys is linked to -PEG2-PEG2-γGlu-CO(CH2)16CO2H

SEQ ID NO: 6 - protein, 40 aa, Artificial Sequence; identical to SEQ ID NO: 3
  Polypeptide compound
  MISC_FEATURE (2)..(2): Xaa=Aib
  MISC_FEATURE (10)..(10): A side chain of Lys is linked to -PEG2-PEG2-γGlu-CO(CH2)14CH3

SEQ ID NO: 7 - protein, 40 aa, Artificial Sequence
  Polypeptide compound
  MISC_FEATURE (2)..(2): Xaa=D-Ser
  MISC_FEATURE (17)..(17): A side chain of Lys is linked to -PEG2-PEG2-γGlu-CO(CH2)16CO2H
HXQGTFTSDYSKYLDAKAAHDFVEWLLRTGGPSSGAPPPS

SEQ ID NO: 8 - protein, 40 aa, Artificial Sequence
  Polypeptide compound
  MISC_FEATURE (2)..(2): Xaa=D-Ser
  MISC_FEATURE (20)..(20): A side chain of Lys is linked to -PEG2-PEG2-γGlu-CO(CH2)16CO2H
HXQGTFTSDYSKYLDEKAAKEFIEWLLRTGGPSSGAPPPS

SEQ ID NO: 9 - protein, 40 aa, Artificial Sequence
  Polypeptide compound
  MISC_FEATURE (2)..(2): Xaa=D-Ser
  MISC_FEATURE (17)..(17): A side chain of Lys is linked to -PEG2-PEG2-γGlu-CO(CH2)16CO2H
HXQGTFTSDYSKYLDEKAAHDFVEWLLNGGGPSSGAPPPS

SEQ ID NO: 10 - protein, 40 aa, Artificial Sequence
  Polypeptide compound
  MISC_FEATURE (2)..(2): Xaa=D-Ser
  MISC_FEATURE (20)..(20): A side chain of Lys is linked to -PEG2-PEG2-γGlu-CO(CH2)14CH3
HXQGTFTSDYSKYLDEKAAKEFIEWLLRGGGPSSGAPPPS

SEQ ID NO: 11 - protein, 40 aa, Artificial Sequence; identical to SEQ ID NO: 10
  Polypeptide compound
  MISC_FEATURE (2)..(2): Xaa=D-Ser
  MISC_FEATURE (20)..(20): A side chain of Lys is linked to -PEG2-PEG2-γGlu-CO(CH2)16CH3

SEQ ID NO: 12 - protein, 40 aa, Artificial Sequence
  Polypeptide compound
  MISC_FEATURE (2)..(2): Xaa=D-Ser
  MISC_FEATURE (20)..(20): A side chain of Lys is linked to -PEG2-PEG2-γGlu-CO(CH2)16CO2H
HXQGTFTSDYSKYLDEKAAKEFIEWLLNGGGPSSGAPPPS

SEQ ID NO: 13 - protein, 40 aa, Artificial Sequence; identical to SEQ ID NO: 12
  Polypeptide compound
  MISC_FEATURE (2)..(2): Xaa=D-Ser
  MISC_FEATURE (20)..(20): A side chain of Lys is linked to -PEG2-PEG2-γGlu-CO(CH2)14CO2H

SEQ ID NO: 14 - protein, 40 aa, Artificial Sequence; identical to SEQ ID NO: 12
  Polypeptide compound
  MISC_FEATURE (2)..(2): Xaa=D-Ser
  MISC_FEATURE (20)..(20): A side chain of Lys is linked to -PEG2-PEG2-γGlu-CO(CH2)16CH3

SEQ ID NO: 15 - protein, 40 aa, Artificial Sequence; identical to SEQ ID NO: 12
  Polypeptide compound
  MISC_FEATURE (2)..(2): Xaa=D-Ser
  MISC_FEATURE (20)..(20): A side chain of Lys is linked to -PEG2-PEG2-γGlu-CO(CH2)14CH3

SEQ ID NO: 16 - protein, 40 aa, Artificial Sequence
  Polypeptide compound
  MISC_FEATURE (2)..(2): Xaa=D-Ser
  MISC_FEATURE (17)..(17): A side chain of Lys is linked to -PEG2-PEG2-γGlu-CO(CH2)14CH3
HXQGTFTSDYSKYLDKKRAQDFVQWLMNTGGPSSGAPPPS

SEQ ID NO: 17 - protein, 40 aa, Artificial Sequence; identical to SEQ ID NO: 1
  Polypeptide compound
  MISC_FEATURE (2)..(2): Xaa=D-Ser
  MISC_FEATURE (16)..(16): A side chain of Lys is linked to -PEG2-PEG2-γGlu-CO(CH2)16CO2H

SEQ ID NO: 18 - protein, 40 aa, Artificial Sequence; identical to SEQ ID NO: 1
  Polypeptide compound
  MISC_FEATURE (2)..(2): Xaa=D-Ser
  MISC_FEATURE (16)..(16): A side chain of Lys is linked to -PEG2-PEG2-CO(CH2)16CO2H

SEQ ID NO: 19 - protein, 40 aa, Artificial Sequence; identical to SEQ ID NO: 1
  Polypeptide compound
  MISC_FEATURE (2)..(2): Xaa=D-Ser
  MISC_FEATURE (16)..(16): A side chain of Lys is linked to -PEG2-PEG2-γGlu-CO(CH2)16CH3

SEQ ID NO: 20 - protein, 40 aa, Artificial Sequence
  Polypeptide compound
  MISC_FEATURE (2)..(2): Xaa=D-Ser
  MISC_FEATURE (16)..(16): A side chain of Lys is linked to -PEG2-PEG2-γGlu-CO(CH2)14CH3
  MISC_FEATURE (27)..(27): Xaa=Nle
HXQGTFTSDYSKYLDKRRAQDFVQWLXNTGGPSSGAPPPS

SEQ ID NO: 21 - protein, 40 aa, Artificial Sequence; identical to SEQ ID NO: 20
  Polypeptide compound
  MISC_FEATURE (2)..(2): Xaa=D-Ser
  MISC_FEATURE (16)..(16): A side chain of Lys is linked to -PEG2-PEG2-γGlu-CO(CH2)16CO2H
  MISC_FEATURE (27)..(27): Xaa=Nle

SEQ ID NO: 22 - protein, 40 aa, Artificial Sequence
  Polypeptide compound
  MISC_FEATURE (2)..(2): Xaa=D-Ser
  MISC_FEATURE (16)..(16): A side chain of Lys is linked to -PEG2-PEG2-γGlu-CO(CH2)16CO2H
HXQGTFTSDYSKYLDKRRAQDFVQWLLNTGGPSSGAPPPS

SEQ ID NO: 23 - protein, 40 aa, Artificial Sequence; identical to SEQ ID NO: 22
  Polypeptide compound
  MISC_FEATURE (2)..(2): Xaa=D-Ser
  MISC_FEATURE (16)..(16): A side chain of Lys is linked to -PEG2-PEG2-γGlu-CO(CH2)14CH3

SEQ ID NO: 24 - protein, 40 aa, Artificial Sequence; identical to SEQ ID NO: 20
  Polypeptide compound
  MISC_FEATURE (2)..(2): Xaa=D-Ser
  MISC_FEATURE (16)..(16): A side chain of Lys is linked to -PEG2-PEG2-CO(CH2)16CO2H
  MISC_FEATURE (27)..(27): Xaa=Nle

SEQ ID NO: 25 - protein, 40 aa, Artificial Sequence; identical to SEQ ID NO: 22
  Polypeptide compound
  MISC_FEATURE (2)..(2): Xaa=D-Ser
  MISC_FEATURE (16)..(16): A side chain of Lys is linked to -PEG2-PEG2-CO(CH2)14CH3

SEQ ID NO: 26 - protein, 40 aa, Artificial Sequence
  Polypeptide compound
  MISC_FEATURE (2)..(2): Xaa = Aib or D-Ser
  MISC_FEATURE (10)..(10): Xaa=Lys or Tyr
  MISC_FEATURE (13)..(13): Xaa=Lys or Tyr
  MISC_FEATURE (16)..(16): Xaa= Glu or Lys
  MISC_FEATURE (17)..(17): Xaa=Lys or Arg
  MISC_FEATURE (18)..(18): Xaa=Arg or Ala
  MISC_FEATURE (20)..(20): Xaa=His，Gln or Lys
  MISC_FEATURE (21)..(21): Xaa=Asp or Glu
  MISC_FEATURE (23)..(23): Xaa= IIe or Val
  MISC_FEATURE (24)..(24): Xaa=Glu or Gln
  MISC_FEATURE (27)..(27): Xaa=Met，Leu or Nle
  MISC_FEATURE (28)..(28): Xaa=Asn，Asp or Arg
  MISC_FEATURE (29)..(29): Xaa=Gly or Thr
HXQGTFTSDXSKXLDXXXAXXFXXWLXXXGGPSSGAPPPS